European Patent Application EP 4 190 329 A1, published June 7, 2023. Title: COLD MEDICINE AND ANTIVIRAL MEDICINE. Applicant: OTSUKA PHARMACEUTICAL FACTORY, INC. The sequence listing filed with the application follows.

SEQUENCE LISTING (6 sequences)

SEQ ID NO: 1 - DNA, 20 bp, artificial
  primer
cagtcaaatgggctgatgca

SEQ ID NO: 2 - DNA, 29 bp, artificial
  primer
aaagggctataaagagaataaggtattct

SEQ ID NO: 3 - DNA, 24 bp, artificial
  probe
ccctgacgaccacgttgtggttca

SEQ ID NO: 4 - DNA, 23 bp, artificial
  primer
cgatgaggctattccgactaggt

SEQ ID NO: 5 - DNA, 27 bp, artificial
  primer
ccttcctgagccttcaatatagtaacc

SEQ ID NO: 6 - DNA, 22 bp, artificial
  probe
tccgcctggcacggtactccct